European Patent Application EP 4 640 824 A2, published October 29, 2025. Title: Methods of Genomic Evaluation in Livestock. Applicant: Inguran, LLC. Application EP. The sequence listing filed with the application follows.

SEQUENCE LISTING (4 sequences)

SEQ ID NO: 1 - DNA, 21 bp, Bos taurus
  source 1..21: mol_type = genomic DNA
gaggctattcggctatgactg

SEQ ID NO: 2 - DNA, 21 bp, Bos taurus
  source 1..21: mol_type = genomic DNA
tcgacaagaccggcttccatc

SEQ ID NO: 3 - DNA, 30 bp, Bos taurus
  source 1..30: mol_type = genomic DNA
aggtcgcgagattggtcgctaggtcatgca

SEQ ID NO: 4 - DNA, 29 bp, Bos taurus
  source 1..29: mol_type = genomic DNA
aagacctcgagagaccctcttcaacacgt